European Patent Application EP 4 205 847 A1, published July 5, 2023. Title: Heterojunction photocatalyst, photocatalyst composite, method for producing heterojunction photocatalyst, and method for producing hydrogen. Applicant: Kao Corporation. The sequence listing filed with the application follows.

SEQUENCE LISTING (17 sequences)

SEQ ID NO: 1 - DNA, 555 bp, Artificial Sequence
  TiBP-DPS-AgBP DNA
aaggagatatacataatgcgcaaactgccggatgcgaaaaccattaatagcgttgataccaaagaatttctgaaccatcaggtggccaatctgaatgtttttaccgtgaaaatccatcagatccactggtatatgcgtggccataacttttttaccctgcacgaaaaaatggatgatctgtatagcgaatttggcgagcagatggatgaagttgcagaacgtctgctggcaattggtggtagcccgtttagcaccctgaaagagtttctggaaaacgcaagcgttgaagaagcaccgtataccaaaccgaaaaccatggatcaactgatggaagatctggttggcaccctggaactgctgcgtgatgaatataaacagggtattgaactgaccgataaagaaggtgacgacgttaccaatgatatgctgattgcatttaaagccagcatcgataaacacatctggatgtttaaagcctttctgggtaaagcaccgctggaaagcctggcgacccagccgcctcgcacgccaccggtgtaaagcttgcggccgcac

SEQ ID NO: 2 - protein, 173 aa, Artificial Sequence
  TiBP-DPS-AgBP AA
RKLPDAKTINSVDTKEFLNHQVANLNVFTVKIHQIHWYMRGHNFFTLHEKMDDLYSEFGEQMDEVAERLLAIGGSPFSTLKEFLENASVEEAPYTKPKTMDQLMEDLVGTLELLRDEYKQGIELTDKEGDDVTNDMLIAFKASIDKHIWMFKAFLGKAPLESLATQPPRTPPV

SEQ ID NO: 3 - protein, 12 aa, Artificial Sequence
  aptamer having high adsorption performance for the solid mediator Ag
AYSSGAPPMPPF

SEQ ID NO: 4 - protein, 12 aa, Artificial Sequence
  aptamer having high adsorption performance for the solid mediator Ag
SLATQPPRTPPV

SEQ ID NO: 5 - protein, 12 aa, Artificial Sequence
  aptamer having high adsorption performance for the solid mediator Ag
WSWRSPTPHVVT

SEQ ID NO: 6 - protein, 12 aa, Artificial Sequence
  aptamer having high adsorption performance for the solid mediator Ag
MHPKPTPHVVLK

SEQ ID NO: 7 - protein, 12 aa, Artificial Sequence
  aptamer having high adsorption performance for the solid mediator Ag
TMHPRHIQIYPA

SEQ ID NO: 8 - protein, 12 aa, Artificial Sequence
  aptamer having high adsorption performance for the solid mediator Ag
HPVQSTTKWSHI

SEQ ID NO: 9 - protein, 14 aa, Artificial Sequence
  aptamer having high adsorption performance for the solid mediator Au
MHGKTQATSGTIQS

SEQ ID NO: 10 - protein, 17 aa, Artificial Sequence
  aptamer having high adsorption performance for the solid mediator Au
LGQSGQSLQGSEKLTNG

SEQ ID NO: 11 - protein, 15 aa, Artificial Sequence
  aptamer having high adsorption performance for the solid mediator Au
EKLVRGMEGASLHPA

SEQ ID NO: 12 - protein, 12 aa, Artificial Sequence
  aptamer having high adsorption performance for the hydrogen-evolution photocatalyst titanium oxide
RKLPDAPGMHTW

SEQ ID NO: 13 - protein, 12 aa, Artificial Sequence
  aptamer having high adsorption performance for the hydrogen-evolution photocatalyst titanium oxide
QPYLFATDSLIK

SEQ ID NO: 14 - protein, 12 aa, Artificial Sequence
  aptamer having high adsorption performance for the hydrogen-evolution photocatalyst titanium oxide
GHTHYHAVRTQT

SEQ ID NO: 15 - protein, 12 aa, Artificial Sequence
  aptamer having high adsorption performance for the hydrogen-evolution photocatalyst titanium oxide
HEHPSRHHTHHR

SEQ ID NO: 16 - protein, 12 aa, Artificial Sequence
  aptamer having high adsorption performance for the hydrogen-evolution photocatalyst titanium oxide
HHHHISHSLQLV

SEQ ID NO: 17 - protein, 12 aa, Artificial Sequence
  aptamer having high adsorption performance for the hydrogen-evolution photocatalyst titanium oxide
THHKHKPVTQFS